European Patent Application EP 4 464 714 A1, published November 20, 2024. Title: SCREENING METHOD FOR CELL-REPELLING PEPTIDES. Applicant: Karlsruher Institut fuer Technologie. The sequence listing filed with the application follows.

SEQUENCE LISTING (37 sequences)

SEQ ID NO: 1 - skipped

SEQ ID NO: 2 - protein, 9 aa, unidentified
PNATEASKP

SEQ ID NO: 3 - skipped

SEQ ID NO: 4 - protein, 9 aa, unidentified
AIHKWDKKN

SEQ ID NO: 5 - protein, 9 aa, unidentified
SVLNSNAIK

SEQ ID NO: 6 - protein, 5 aa, unidentified
VSAAP

SEQ ID NO: 7 - protein, 12 aa, unidentified
TLSSKMYHTKGQ

SEQ ID NO: 8 - protein, 11 aa, unidentified
WSKICKPVLKE

SEQ ID NO: 9 - protein, 8 aa, unidentified
AEEALPKK

SEQ ID NO: 10 - protein, 8 aa, unidentified
VRSSSRTP

SEQ ID NO: 11 - protein, 16 aa, unidentified
SDKKPVAHVVANPQAE

SEQ ID NO: 12 - protein, 5 aa, unidentified
YQTKV

SEQ ID NO: 13 - protein, 14 aa, unidentified
PCQRETPEGAEAKP

SEQ ID NO: 14 - protein, 15 aa, unidentified
CASEFALRMKIKEVK

SEQ ID NO: 15 - protein, 15 aa, unidentified
ASEFALRMKIKEVKK

SEQ ID NO: 16 - protein, 15 aa, unidentified
SEFALRMKIKEVKKE

SEQ ID NO: 17 - protein, 15 aa, unidentified
EFALRMKIKEVKKEN

SEQ ID NO: 18 - protein, 15 aa, unidentified
FALRMKIKEVKKENG

SEQ ID NO: 19 - protein, 15 aa, unidentified
ALRMKIKEVKKENGD

SEQ ID NO: 20 - protein, 15 aa, unidentified
LRMKIKEVKKENGDK

SEQ ID NO: 21 - protein, 15 aa, unidentified
RMKIKEVKKENGDKK

SEQ ID NO: 22 - protein, 15 aa, unidentified
MKIKEVKKENGDKKI

SEQ ID NO: 23 - protein, 15 aa, unidentified
KIKEVKKENGDKKIV

SEQ ID NO: 24 - protein, 15 aa, unidentified
IKEVKKENGDKKIVP

SEQ ID NO: 25 - protein, 15 aa, unidentified
KEVKKENGDKKIVPK

SEQ ID NO: 26 - protein, 15 aa, unidentified
EVKKENGDKKIVPKK

SEQ ID NO: 27 - protein, 15 aa, unidentified
HPGSAVSASNAIKNL

SEQ ID NO: 28 - protein, 15 aa, unidentified
TPPNATEASKPQGTT

SEQ ID NO: 29 - protein, 15 aa, unidentified
AIKNLPPPTKGQEGS

SEQ ID NO: 30 - protein, 5 aa, unidentified
QETWF

SEQ ID NO: 31 - protein, 8 aa, unidentified
QNGNQGKN

SEQ ID NO: 32 - protein, 15 aa, unidentified
IAMTPPNATEASKPQ

SEQ ID NO: 33 - protein, 15 aa, unidentified
FLCSLFAPVCLDRPI

SEQ ID NO: 34 - protein, 15 aa, unidentified
KENGDKKIVPKKKKP

SEQ ID NO: 35 - protein, 13 aa, unidentified
QETWFQNGWQGKN

SEQ ID NO: 36 - protein, 14 aa, unidentified
QETWFQNGWQGKNP

SEQ ID NO: 37 - protein, 14 aa, unidentified
KEQWFGNRWHEGYR